European Patent Specification EP 3 468 587 B1, published August 26, 2026. Title: Monoclonal Antibodies, Compositions and Methods for Detecting Mucin-like Protein (MLP) as a Marker for Ovarian and Pancreatic Cancer. Applicant: University of Leicester Omeros Corporation Schwaeble, Hans-Wilhelm Demopulos, Gregory A. The sequence listing filed with the application follows.

SEQUENCE LISTING (36 sequences)

SEQ ID NO: 1 - protein, 431 aa, Homo sapiens
MKPRQKEQDTRLRKLRESSEGDQWLENEKTKPLRPQQQPQCQPAGGTGQRRGSGSSPSADQQGAQDREEEAAAAPAPTSRGHRTEKRKPQQPQRRPAGGTGQRRGSRSSSSADQQGAQDREEEAAAAPAPTSSGHRTEKRKPQQPQCRPAAGTGQRRGSGCSPSADQQRAQDREEEATAAPVPTSSGHRTEKRKRLQLQCQPAGGTGQRRGSRSSPSADQQRAQDREEEAAAAPAPTSRGHRTEKRKPQQPQRRPAAGTGQRRGSGCSPSADQQGAQDREEEAAAAPAPTSRGHRTEKRKRLQPQRRPAGGTGQRRGSRSSPSADQQRAQDREEEAAAAPVPTSRGHRTEKRKRLQLQCQPAGGTGQRRGSGSSPSADQQRAQDREEEAAAAPAPTSSGHRTEKRKRQQPQRRPAAGTGQRRGSEEMEEEG

SEQ ID NO: 2 - DNA, 971 bp, Artificial
  Synthetic
attttgtttactttaagaaggagatatacatatgcggggttctcatcatcatcatcatcatggtatggctagcatgactggtggacagcaaatgggtcgggatctgtacgacgatgacgataaggatcgatggggatcccccgggctgcaggaattcggcacgagagaagaggaagccgcagcagccccagcgccgaccagcagggggcacaggacagagaagaggaagcggctacagccccagcgccgaccagcagggggcacaggacagagaagaggaagccgcagcagccccagcgccgaccagcagcgggcacaggacagagaagaggaagcggctgcagctccagtgccaaccagcagggggcacaggacagagaagaggaagcggctgcagctccagtgccaaccagcagggggcacaggacagagaagaggaagcggcagcagccccagtgccgaccagcagcgggcacaggacagagaagaggaagccgcagcagccccagcgccgaccagcagcgggcacaggacagagaagaggaagcggcagcagccccagcgccgaccagcagcgggcacaggacagagaagaggaagtgaggaaatggaagaagagggttgacctgagctgaaggacatgaacttccacgtgaaatagccccagggccgggcacacgaggtcaggagttcaagaccagcctggccaagatggtgaaaccctgtctctactaaaaataaaaaattagctgggtgcggtggcaggcacctgtaatcccagctactcaggaggctgaggcaggagaatcacttgaacccaggaggtggaggttacagtgagccaagatctcaccactgcactgtagcctgggcaacagagcaagactccatgaaaaaaaaaaaaaaaaactcgagggggggcccggtaccatggaattcgaagcttgatccggctgctaacaaagcccgaa

SEQ ID NO: 3 - protein, 197 aa, Artificial
  Synthetic
MRGSHHHHHHGMASMTGGQQMGRDLYDDDDKDRWGSPGLQEFGTREEEAAAAPAPTSRGHRTEKRKRLQPQRRPAGGTGQRRGSRSSPSADQQRAQDREEEAAAAPVPTSRGHRTEKRKRLQLQCQPAGGTGQRRGSGSSPSADQQRAQDREEEAAAAPAPTSSGHRTEKRKRQQPQRRPAAGTGQRRGSEEMEEEG

SEQ ID NO: 4 - protein, 153 aa, Artificial
  Synthetic
REEEAAAAPAPTSRGHRTEKRKRLQPQRRPAGGTGQRRGSRSSPSADQQRAQDREEEAAAAPVPTSRGHRTEKRKRLQLQCQPAGGTGQRRGSGSSPSADQQRAQDREEEAAAAPAPTSSGHRTEKRKRQQPQRRPAAGTGQRRGSEEMEEEG

SEQ ID NO: 5 - protein, 35 aa, Artificial
  Synthetic
SSGHRTEKRKRQQPQRRPAAGTGQRRGSEEMEEEG

SEQ ID NO: 6 - protein, 29 aa, Artificial
  Synthetic
EKRKRQQPQRRPAAGTGQRRGSEEMEEEG

SEQ ID NO: 7 - protein, 123 aa, Artificial
  Synthetic
EVQLQQSGPELVKPGASVKISCKASGYAFTGFYIHWMKQSHVKSLEWIGRIHPYNGATSYNQNFKDRASLTVDESSSTAYMEFYGLTSEDSAVYYCARERVYYYGSTYEFDSWGQGTTLTVSS

SEQ ID NO: 8 - protein, 123 aa, Artificial
  Synthetic
EVQLQQSGPELVKPGASVKISCKASGYSFTGFYIHWVKQSHVKSLEWIGRIHPYNGAPTYNQNFKDRARLTVHESSSTAYMEFFGLTSEDSAVYYCARERVYYYGSTYEFDFWGQGTTLTVSS

SEQ ID NO: 9 - protein, 122 aa, Artificial
  Synthetic
DVKLQESGGGLVQPGGSMKLSCVASGFTFSNYWMNWVRQSPEKGLEWVAEIRLKSNNYAINYAESVKGRFTISRDDSKSSVYLDMNNLRAEDTGIYYCTSYYGSSLYYLDYWGQGTTLTVSS

SEQ ID NO: 10 - protein, 112 aa, Artificial
  Synthetic
DVLMTQTPLSLPVSLGDQASISCRSGQSIVHTSGVTYLSWYLQKPGQSPKLLIYKVFYRFSGVPDRFSGSGSGTDFTLKISRVESEDLGVYYCFQGSHVPPTFGAGTKLELK

SEQ ID NO: 11 - protein, 112 aa, Artificial
  Synthetic
DVLMTQTPLSLPVSLGDQASISCRSGQSIVHSSGVTYLSWYLQKPGQSPKLLIYKVFYRFSGVPDRFSGSGSGTDFTLKISRVEAEDLGVYYCFQGSHVPPTFGTGTKLELK

SEQ ID NO: 12 - protein, 106 aa, Artificial
  Synthetic
QIVLTQSPVIMSASPGEKVTISCSASSSVSNMYWYQQKPGSSPKAWIYRTSNLASGVPARFSGSGSGTSYSLTISSMEAEDAATYYCHQYQSYPRTFGAGTKLEIK

SEQ ID NO: 13 - protein, 5 aa, Artificial
  Synthetic
GFYIH

SEQ ID NO: 14 - protein, 17 aa, Artificial
  Synthetic
RIHPYNGATSYNQNFKD

SEQ ID NO: 15 - protein, 14 aa, Artificial
  Synthetic
ERVYYYGSTYEFDS

SEQ ID NO: 16 - protein, 17 aa, Artificial
  Synthetic
RIHPYNGAPTYNQNFKD

SEQ ID NO: 17 - protein, 5 aa, Artificial
  Synthetic
NYWMN

SEQ ID NO: 18 - protein, 19 aa, Artificial
  Synthetic
EIRLKSNNYAINYAESVKG

SEQ ID NO: 19 - protein, 11 aa, Artificial
  Synthetic
YYGSSLYYLDY

SEQ ID NO: 20 - protein, 17 aa, Artificial
  Synthetic
  MISC_FEATURE (9)..(9): Wherein Xaa at position 9 is T or P
  MISC_FEATURE (10)..(10): Wherein Xaa at position 10 is S or T
RIHPYNGAXXYNQNFKD

SEQ ID NO: 21 - protein, 16 aa, Artificial
  Synthetic
RSGQSIVHTSGVTYLS

SEQ ID NO: 22 - protein, 7 aa, Artificial
  Synthetic
KVFYRFS

SEQ ID NO: 23 - protein, 9 aa, Artificial
  Synthetic
FQGSHVPPT

SEQ ID NO: 24 - protein, 16 aa, Artificial
  Synthetic
RSGQSIVHSSGVTYLS

SEQ ID NO: 25 - protein, 10 aa, Artificial
  Synthetic
SASSSVSNMY

SEQ ID NO: 26 - protein, 7 aa, Artificial
  Synthetic
RTSNLAS

SEQ ID NO: 27 - protein, 9 aa, Artificial
  Synthetic
HQYQSYPRT

SEQ ID NO: 28 - protein, 16 aa, Artificial
  Synthetic
  MISC_FEATURE (9)..(9): Wherein Xaa at position 9 is T or S
RSGQSIVHXSGVTYLS

SEQ ID NO: 29 - DNA, 370 bp, Artificial
  Synthetic
gaggtccagctgcaacagtctggacctgagctggtgaagcctggggcttcagtgaagatatcctgcaaggcttctggttacgcattcactggcttctacatacactggatgaagcaaagccatgtaaagagccttgagtggattggacgtattcatccttacaatggtgctactagctataatcagaatttcaaggacagggccagcttgactgtagatgagtcctccagtacagcctacatggagttctatggcctgacatctgaggactctgcagtctattactgtgcaagagagagagtctattactacggtagtacttacgagtttgactcctggggccaaggcaccactctcacagtctcctcag

SEQ ID NO: 30 - DNA, 370 bp, Artificial
  Synthetic
gaggtccagctgcaacaatctggacctgagctggtgaagcctggggcttcagtgaagatatcctgcaaggcttctggttactcattcactggcttctacatacactgggtgaagcaaagccatgtaaagagccttgagtggattggacgtattcatccttacaatggtgctcctacctacaaccagaatttcaaggacagggcccgcttgactgtacatgagtcctccagcacagcctacatggagttctttggcctgacatctgaggactctgcagtctattactgtgcaagagagagagtctattactacggtagtacttacgagtttgacttctggggccaaggcaccactctcacagtctcctcag

SEQ ID NO: 31 - DNA, 367 bp, Artificial
  Synthetic
gatgtgaagcttcaggagtctggaggaggcttggtgcaacctggaggatccatgaaactctcctgtgttgcctctggattcactttcagtaactactggatgaactgggtccgccagtctccagagaaggggcttgagtgggttgctgaaattagattgaaatctaataattatgcaataaattatgcggagtctgtgaaagggaggtttaccatctcaagagatgattccaaaagcagtgtctacctggacatgaacaacttaagagctgaagacactggcatttattactgtacctcctactacggcagtagcctctactaccttgactactggggccaaggcaccactctcacagtctcctcag

SEQ ID NO: 32 - DNA, 337 bp, Artificial
  Synthetic
gatgttttgatgacccaaactccactctccctgcctgtcagtcttggagatcaagcctccatctcttgcagatctggtcagagcattgtccatactagtggcgtcacctatttatcatggtacctgcagaaaccaggccagtctccaaagctcctgatctacaaagttttctaccgattttctggggtcccggacaggttcagtggcagtggatcagggacagatttcacactcaagatcagcagagtggagtctgaggatctgggagtttattactgctttcaaggttcacatgttcctcccacgttcggtgctgggaccaagctggagctgaaac

SEQ ID NO: 33 - DNA, 337 bp, Artificial
  Synthetic
gatgttttgatgacccaaactccactctccctgcctgtcagtcttggagatcaagcctccatctcttgcagatctggtcagagcattgtccatagtagtggcgtcacctatttatcatggtacctgcagaaaccaggccagtctccaaagctcctgatctacaaagttttctaccgattttctggggtcccggacaggttcagtggcagtggatcagggacagatttcacactcaagatcagcagagtggaggctgaggatctgggagtttattactgctttcagggttcacatgttcctcccacgttcggtactgggaccaagctggagctgaaac

SEQ ID NO: 34 - DNA, 319 bp, Artificial
  Synthetic
caaattgttctcacccagtctccagtaatcatgtctgcatctccaggggagaaggtcaccatatcctgcagtgccagctcaagtgtaagtaacatgtactggtaccagcagaagccaggatcctcccccaaagcctggatttatcgcacatccaacctggcttctggagtccctgctcgcttcagtggcagtgggtctgggacctcttactctctcacaatcagcagcatggaggctgaagatgctgccacttattactgccaccagtatcaaagttacccacggacgttcggtgcaggcaccaagctggaaatcaaac

SEQ ID NO: 35 - protein, 14 aa, Artificial
  Synthetic
ERVYYYGSTYEFDF

SEQ ID NO: 36 - protein, 14 aa, Artificial
  Synthetic
  MISC_FEATURE (14)..(14): Wherein Xaa at position 14 is S or F
ERVYYYGSTYEFDX